European Patent Application EP 4 435 116 A2, published September 25, 2024. Title: SECOND STRAND DIRECT. Applicant: Bio-Rad Laboratories, Inc. Application EP. The sequence listing filed with the application follows.

SEQUENCE LISTING (39 sequences)

SEQ ID NO: 1 - DNA, 31 bp, synthetic construct
  misc_feature 1..31: note = synthetic nucleotide sequence
  source 1..31: mol_type = other DNA
aatgagatacggcgaccaccgagatctacac

SEQ ID NO: 2 - DNA, 24 bp, synthetic construct
  misc_feature 1..24: note = synthetic nucleotide sequence
  source 1..24: mol_type = other DNA
caagcagaagacggcatacgagat

SEQ ID NO: 3 - DNA, 51 bp, synthetic construct
  misc_feature 1..51: note = synthetic nucleotide sequence
  misc_feature 25..28: note = n is a, c, g, or t
  misc_feature 29..36: note = n is a, c, g, or t; "n" may be present or absent
  source 1..51: mol_type = other DNA
caagcagaagacggcatacgagatnnnnnnnnnnnngtctcgtgggctcgg

SEQ ID NO: 4 - DNA, 50 bp, synthetic construct
  misc_feature 1..50: note = synthetic nucleotide sequence
  misc_feature 25..28: note = n is a, c, g, or t
  misc_feature 29..36: note = n is a, c, g, or t; "n" may be present or absent
  source 1..50: mol_type = other DNA
caagcagaagacggcatacgagatnnnnnnnnnnnntcgtcggcagcgtc

SEQ ID NO: 5 - DNA, 58 bp, synthetic construct
  misc_feature 1..58: note = synthetic nucleotide sequence
  misc_feature 32..35: note = n is a, c, g, or t
  misc_feature 36..43: note = n is a, c, g, or t; "n" may be present or absent
  source 1..58: mol_type = other DNA
aatgagatacggcgaccaccgagatctacacnnnnnnnnnnnngtctcgtgggctcgg

SEQ ID NO: 6 - DNA, 57 bp, synthetic construct
  misc_feature 1..57: note = synthetic nucleotide sequence
  misc_feature 32..35: note = n is a, c, g, or t
  misc_feature 36..43: note = n is a, c, g, or t; "n" may be present or absent
  source 1..57: mol_type = other DNA
aatgagatacggcgaccaccgagatctacacnnnnnnnnnnnntcgtcggcagcgtc

SEQ ID NO: 7 - DNA, 15 bp, synthetic construct
  misc_feature 1..15: note = synthetic nucleotide sequence
  source 1..15: mol_type = other DNA
gtctcgtgggctcgg

SEQ ID NO: 8 - DNA, 14 bp, synthetic construct
  misc_feature 1..14: note = synthetic nucleotide sequence
  source 1..14: mol_type = other DNA
tcgtcggcagcgtc

SEQ ID NO: 9 - DNA, 37 bp, synthetic construct
  misc_feature 1..37: note = synthetic nucleotide sequence
  source 1..37: mol_type = other DNA
gcctgtccgcggaagcagtggtatcaacgcagagtac

SEQ ID NO: 10 - DNA, 19 bp, synthetic construct
  misc_feature 1..19: note = synthetic nucleotide sequence
  source 1..19: mol_type = other DNA
agatgtgtataagagacag

SEQ ID NO: 11 - DNA, 19 bp, synthetic construct
  misc_feature 1..19: note = synthetic nucleotide sequence
  source 1..19: mol_type = other DNA
agatgtgtataagagacag

SEQ ID NO: 12 - DNA, 34 bp, synthetic construct
  misc_feature 1..34: note = synthetic nucleotide sequence
  source 1..34: mol_type = other DNA
gtctcgtgggctcggagatgtgtataagagacag

SEQ ID NO: 13 - DNA, 19 bp, synthetic construct
  misc_feature 1..19: note = synthetic nucleotide sequence
  source 1..19: mol_type = other DNA
ctgtctcttatacacatct

SEQ ID NO: 14 - DNA, 33 bp, synthetic construct
  misc_feature 1..33: note = synthetic nucleotide sequence
  source 1..33: mol_type = other DNA
acactctttccctacacgacgctcttccgatct

SEQ ID NO: 15 - DNA, 29 bp, synthetic construct
  misc_feature 1..29: note = synthetic nucleotide sequence
  source 1..29: mol_type = other DNA
aatgatacggcgaccaccgagatctacac

SEQ ID NO: 16 - DNA, 56 bp, synthetic construct
  misc_feature 1..56: note = synthetic nucleotide sequence
  misc_feature 30..33: note = n is a, c, g, or t
  misc_feature 34..41: note = n is a, c, g, or t; "n" may be present or absent
  source 1..56: mol_type = other DNA
aatgatacggcgaccaccgagatctacacnnnnnnnnnnnngtctcgtgggctcgg

SEQ ID NO: 17 - DNA, 55 bp, synthetic construct
  misc_feature 1..55: note = synthetic nucleotide sequence
  misc_feature 30..33: note = n is a, c, g, or t
  misc_feature 34..41: note = n is a, c, g, or t; "n" may be present or absent
  source 1..55: mol_type = other DNA
aatgatacggcgaccaccgagatctacacnnnnnnnnnnnntcgtcggcagcgtc

SEQ ID NO: 18 - DNA, 33 bp, synthetic construct
  misc_feature 1..33: note = synthetic nucleotide sequence
  source 1..33: mol_type = other DNA
tcgtcggcagcgtcagatgtgtataagagacag

SEQ ID NO: 19 - DNA, 70 bp, synthetic construct
  misc_feature 1..70: note = synthetic nucleotide sequence
  misc_feature 25..28: note = n is a, c, g, or t
  misc_feature 29..36: note = n is a, c, g, or t; "n" may be present or absent
  source 1..70: mol_type = other DNA
caagcagaagacggcatacgagatnnnnnnnnnnnngtctcgtgggctcggagatgtgtataagagacag

SEQ ID NO: 20 - DNA, 74 bp, synthetic construct
  misc_feature 1..74: note = synthetic nucleotide sequence
  misc_feature 30..33: note = n is a, c, g, or t
  misc_feature 34..41: note = n is a, c, g, or t; "n" may be present or absent
  source 1..74: mol_type = other DNA
aatgatacggcgaccaccgagatctacacnnnnnnnnnnnntcgtcggcagcgtcagatgtgtataagagacag

SEQ ID NO: 21 - DNA, 48 bp, synthetic construct
  misc_feature 1..48: note = synthetic nucleotide sequence
  source 1..48: mol_type = other DNA
tcgtcggcagcgtcagatgtgtataagagagatgtgtataagagacag

SEQ ID NO: 22 - DNA, 29 bp, synthetic construct
  misc_feature 1..29: note = synthetic nucleotide sequence
  source 1..29: mol_type = other DNA
tcgtcggcagcgtcagatgtgtataagag

SEQ ID NO: 23 - DNA, 57 bp, synthetic construct
  misc_feature 1..57: note = synthetic nucleotide sequence
  source 1..57: mol_type = other DNA
aatgatacggcgaccaccgagatctacatcgtcggcacgctcagatgtgtataagag

SEQ ID NO: 24 - DNA, 73 bp, synthetic construct
  misc_feature 1..73: note = synthetic nucleotide sequence
  misc_feature 34..37: note = n is a, c, g, or t
  misc_feature 38..45: note = n is a, c, g, or t; "n" may be present or absent
  source 1..73: mol_type = other DNA
ctgtctcttatacacatctgacgctgccgacgannnnnnnnnnnngtgtagtctcggtggtcgccgtatcatt

SEQ ID NO: 25 - DNA, 70 bp, synthetic construct
  misc_feature 1..70: note = synthetic nucleotide sequence
  misc_feature 25..28: note = n is a, c, g, or t
  misc_feature 29..36: note = n is a, c, g, or t; "n" may be present or absent
  source 1..70: mol_type = other DNA
caagcagaagacggcatacgagatnnnnnnnnnnnngtctcgtgggctcggagatgtgtataagagagag

SEQ ID NO: 26 - DNA, 69 bp, synthetic construct
  misc_feature 1..69: note = synthetic nucleotide sequence
  misc_feature 35..38: note = n is a, c, g, or t
  misc_feature 39..46: note = n is a, c, g, or t; "n" may be present or absent
  source 1..69: mol_type = other DNA
ctgtctcttatacacatctccgagcccacgagacnnnnnnnnnnnnatctcgtatgccgcttctgcttg

SEQ ID NO: 27 - DNA, 49 bp, synthetic construct
  misc_feature 1..49: note = synthetic nucleotide sequence
  misc_feature 24..27: note = n is a, c, g, or t
  misc_feature 28..35: note = n is a, c, g, or t; "n" may be present or absent
  source 1..49: mol_type = other DNA
caagcagaagacggatacgagatnnnnnnnnnnnntcgtcggcagcgtc

SEQ ID NO: 28 - DNA, 68 bp, synthetic construct
  misc_feature 1..68: note = synthetic nucleotide sequence
  misc_feature 25..28: note = n is a, c, g, or t
  misc_feature 29..36: note = n is a, c, g, or t; "n" may be present or absent
  source 1..68: mol_type = other DNA
caagcagaagacggcatacgagatnnnnnnnnnnnntcgtcggcagcgtcagatgtgtataagaacag

SEQ ID NO: 29 - DNA, 68 bp, synthetic construct
  misc_feature 1..68: note = synthetic nucleotide sequence
  misc_feature 34..37: note = n is a, c, g, or t
  misc_feature 38..45: note = n is a, c, g, or t; "n" may be present or absent
  source 1..68: mol_type = other DNA
ctgtctcttatacacatctgacgctgccgacgannnnnnnnnnnnatctcgtatgccgcttctgcttg

SEQ ID NO: 30 - DNA, 56 bp, synthetic construct
  misc_feature 1..56: note = synthetic nucleotide sequence
  misc_feature 25..28: note = n is a, c, g, or t
  misc_feature 29..36: note = n is a, c, g, or t; "n" may be present or absent
  source 1..56: mol_type = other DNA
caagcagaagacggcatacgagatnnnnnnnnnnnngtctcgtgggctcggctcgg

SEQ ID NO: 31 - DNA, 69 bp, synthetic construct
  misc_feature 1..69: note = synthetic nucleotide sequence
  misc_feature 25..28: note = n is a, c, g, or t
  misc_feature 29..36: note = n is a, c, g, or t; "n" may be present or absent
  source 1..69: mol_type = other DNA
caagcagaagacggcatacgagatnnnnnnnnnnnngtctcgtgggctcggagatgtgtataagagcag

SEQ ID NO: 32 - DNA, 66 bp, synthetic construct
  misc_feature 1..66: note = synthetic nucleotide sequence
  source 1..66: mol_type = other DNA
aatgatacggcgaccaccgagatctacacgcctgtccgcggaagcagtggtatcaacgcagagtac

SEQ ID NO: 33 - DNA, 69 bp, synthetic construct
  misc_feature 1..69: note = synthetic nucleotide sequence
  misc_feature 25..28: note = n is a, c, g, or t
  misc_feature 29..36: note = n is a, c, g, or t; "n" may be present or absent
  source 1..69: mol_type = other DNA
caagcagaagacggcatacgagatnnnnnnnnnnnntcgtcggcagcgtcagatgtgtataagagacag

SEQ ID NO: 34 - DNA, 69 bp, synthetic construct
  misc_feature 1..69: note = synthetic nucleotide sequence
  misc_feature 34..37: note = n is a, c, g, or t
  misc_feature 38..45: note = n is a, c, g, or t; "n" may be present or absent
  source 1..69: mol_type = other DNA
ctgtctcttatacacatctgacgctgccgacgannnnnnnnnnnnatctcgtatgccgtcttctgcttg

SEQ ID NO: 35 - DNA, 70 bp, synthetic construct
  misc_feature 1..70: note = synthetic nucleotide sequence
  misc_feature 35..38: note = n is a, c, g, or t
  misc_feature 39..46: note = n is a, c, g, or t; "n" may be present or absent
  source 1..70: mol_type = other DNA
ctgtctcttatacacatctccgagcccacgagacnnnnnnnnnnnnatctcgtatgccgtcttctgcttg

SEQ ID NO: 36 - DNA, 66 bp, synthetic construct
  misc_feature 1..66: note = synthetic nucleotide sequence
  source 1..66: mol_type = other DNA
gtactctgcgttgataccactgcttccgcggacaggcgtgtagatctcggtggtcgccgtatcatt

SEQ ID NO: 37 - DNA, 34 bp, synthetic construct
  misc_feature 1..34: note = synthetic nucleotide sequence
  source 1..34: mol_type = other DNA
ctgtctcttatacacatctccgagcccacgagac

SEQ ID NO: 38 - DNA, 33 bp, synthetic construct
  misc_feature 1..33: note = synthetic nucleotide sequence
  source 1..33: mol_type = other DNA
ctgtctcttatacacatctgacgctgccgacga

SEQ ID NO: 39 - DNA, 30 bp, synthetic construct
  misc_feature 1..30: note = synthetic nucleotide sequence
  source 1..30: mol_type = other DNA
gtctcgtgggctcggagatgtgtataagag